European Patent Application EP 4 382 166 A1, published June 12, 2024. Title: ANTI-PD-L1 NANOBODY AND USE THEREOF. Applicant: BETTA PHARMACEUTICALS CO., LTD. Application EP 22852325.4, filed August 5, 2022. The sequence listing filed with the application follows.

SEQUENCE LISTING (32 sequences)

SEQ ID NO: 1 - protein, 8 aa, synthetic construct
GRSFSSSG

SEQ ID NO: 2 - protein, 8 aa, synthetic construct
INSSGGDT

SEQ ID NO: 3 - protein, 17 aa, synthetic construct
AAKEGGGPSSIPAIYDY

SEQ ID NO: 4 - protein, 124 aa, synthetic construct
QVQLVESGGGLVQAGGSLRLSCAASGRSFSSSGMGWFRQAPGKDREFVATINSSGGDTYYRDSVEGRFTTSRDNAKNTMSLQMNDLKPEDTAVYYCAAKEGGGPSSIPAIYDYWGQGTQVTVSS

SEQ ID NO: 5 - protein, 8 aa, synthetic construct
GFTFSSYA

SEQ ID NO: 6 - protein, 8 aa, synthetic construct
INTGSEIV

SEQ ID NO: 7 - protein, 12 aa, synthetic construct
ATGLVSAEHDGI

SEQ ID NO: 8 - protein, 119 aa, synthetic construct
QVQLVESGGGLVQPGGSLSLSCVASGFTFSSYAMRWVRQAPGKEPEWVAGINTGSEIVVYANSVRGRFAISRDNARDTLFLQMNSLKPEDTAVYYCATGLVSAEHDGIWGQGTQVTVSS

SEQ ID NO: 9 - protein, 8 aa, synthetic construct
GRDFLTYG

SEQ ID NO: 10 - protein, 8 aa, synthetic construct
INWSGSMT

SEQ ID NO: 11 - protein, 17 aa, synthetic construct
AARRGAVTYASSNEYEH

SEQ ID NO: 12 - protein, 124 aa, synthetic construct
EVQLVESGGGSVQTGGSLRLSCVASGRDFLTYGMGWFRQAPGKEREFVASINWSGSMTYYADSVKGRFTISRDNAKNTVYLQMNSLKPGDTAVYICAARRGAVTYASSNEYEHWGQGTQVTVSS

SEQ ID NO: 13 - protein, 124 aa, synthetic construct
EVQLVESGGGLVQAGDSLRLSCTASGRDFLTYGMGWFRQAPGKEREFVASINWSGSMTYYADSVKGRFTISRDNAKNTVYLQMNSLKPGDTAVYICAARRGAVTYASSNEYEHWGQGTQVTVSS

SEQ ID NO: 14 - protein, 17 aa, synthetic construct
AAKEGGGPSSIPAIFDY

SEQ ID NO: 15 - protein, 124 aa, synthetic construct
QVQLVESGGGLVQAGGSLRLSCAASGRSFSSSGMGWFRQAPGKDREFVATINSSGGDTYYADSVEGRFTTSRDNAKNTMSLQMNDLKPEDTAVYYCAAKEGGGPSSIPAIFDYWGQGTQVTVSS

SEQ ID NO: 16 - protein, 25 aa, synthetic construct
QVQLVESGGGLVQAGGSLRLSCAAS

SEQ ID NO: 17 - protein, 17 aa, synthetic construct
MGWFRQAPGKDREFVAT

SEQ ID NO: 18 - protein, 38 aa, synthetic construct
YYRDSVEGRFTTSRDNAKNTMSLQMNDLKPEDTAVYYC

SEQ ID NO: 19 - protein, 11 aa, synthetic construct
WGQGTQVTVSS

SEQ ID NO: 20 - protein, 25 aa, synthetic construct
QVQLVESGGGLVQPGGSLSLSCVAS

SEQ ID NO: 21 - protein, 17 aa, synthetic construct
MRWVRQAPGKEPEWVAG

SEQ ID NO: 22 - protein, 38 aa, synthetic construct
VYANSVRGRFAISRDNARDTLFLQMNSLKPEDTAVYYC

SEQ ID NO: 23 - protein, 25 aa, synthetic construct
EVQLVESGGGSVQTGGSLRLSCVAS

SEQ ID NO: 24 - protein, 17 aa, synthetic construct
MGWFRQAPGKEREFVAS

SEQ ID NO: 25 - protein, 38 aa, synthetic construct
YYADSVKGRFTISRDNAKNTVYLQMNSLKPGDTAVYIC

SEQ ID NO: 26 - protein, 25 aa, synthetic construct
EVQLVESGGGLVQAGDSLRLSCTAS

SEQ ID NO: 27 - protein, 38 aa, synthetic construct
YYADSVEGRFTTSRDNAKNTMSLQMNDLKPEDTAVYYC

SEQ ID NO: 28 - protein, 124 aa, synthetic construct
QVQLVESGGGVVQPGGSLRLSCAASGRSFSSSGMGWFRQAPGKGREFVATINSSGGDTYYRDSVEGRFTTSRDNSKNTMYLQMNSLRAEDTAVYYCAAKEGGGPSSIPAIYDYWGQGTLVTVSS

SEQ ID NO: 29 - protein, 119 aa, synthetic construct
QVQLVESGGGVVQPGGSLRLSCAASGFTFSSYAMRWVRQAPGKGLEWVAGINTGSEIVVYANSVRGRFTISRDNSRDTLYLQMNSLRAEDTAVYYCATGLVSAEHDGIWGQGTQVTVSS

SEQ ID NO: 30 - protein, 124 aa, synthetic construct
EVQLVESGGGLVQPGGSLRLSCAASGRDFLTYGMGWFRQAPGKGREFVASINWSGSMTYYADSVKGRFTISRDNAKNTVYLQMNSLKAEDTAVYICAARRGAVTYASSNEYEHWGQGTLVTVSS

SEQ ID NO: 31 - protein, 124 aa, synthetic construct
EVQLVESGGGLVQPGGSLRLSCTASGRDFLTYGMGWFRQAPGKELEFVASINWSGSMTYYADSVKGRFTISRDNAKNTVYLQMNSLRAEDTAVYICAARRGAVTYASSNEYEHWGQGTQVTVSS

SEQ ID NO: 32 - protein, 124 aa, synthetic construct
EVQLVESGGGLVQPGGSLRLSCAASGRDFLTYGMGWFRQAPGKGLEFVASINWSGSMTYYADSVKGRFTISRDNAKNSVYLQMNSLRAEDTAVYICAARRGAVTYASSNEYEHWGQGTQVTVSS